European Patent Application EP 4 331 615 A1, published March 6, 2024. Title: ANTIBODY-DRUG CONJUGATE TARGETING NECTIN-4 AND PREPARATION METHOD THEREFOR AND USE THEREOF. Applicant: JIANGSU MABWELL HEALTH PHARMACEUTICAL R&D CO., LTD. MABWELL (SHANGHAI) BIOSCIENCE CO., LTD. The sequence listing filed with the application follows.

SEQUENCE LISTING (20 sequences)

SEQ ID NO: 1 - protein, 119 aa, artificial sequence
  42D20-hz63,VH
QVQLQESGPGLVKPSETLSLTCTVSGFSLIDYGVSWIRQPPGKGLEWIGVIWGGGKIYYNSVLKSRVTISKDNSKSQVSLKLSSVTAADTAVYYCAKQGGLLFYAMDYWGQGTLVTVSS

SEQ ID NO: 2 - protein, 113 aa, artificial sequence
  42D20-hz63, VL
DIVMTQSPDSLAVSLGERATINCKSSQSLLNTYSQKNYLAWYQQKPGQSPKLLIYFASTRESGVPDRFSGSGSETDFTLTISSLQAEDLAVYFCQQHYNTPFTFGAGTKLELK

SEQ ID NO: 3 - protein, 119 aa, artificial sequence
  42D20-hz10, VH
QVQLQESGPGLVKPSETLSLTCTVSGFSLIDYGVSWIRQPPGKGLEWIGVIWGDGKIYYNSVLKSRVTISKDNSKSQVSLKLSSVTAADTAVYYCAKQGGLLFYAMDYWGQGTLVTVSS

SEQ ID NO: 4 - protein, 113 aa, artificial sequence
  42D20-hz10, VL
DIVMTQSPDSLAVSLGERATINCKSSQSLLNSYSQKNYLAWYQQKPGQPPKLLIYFASTRESGVPDRFSGSGSGTDFTLTISSLQAEDVAVYYCQQHYNTPFTFGAGTKLELK

SEQ ID NO: 5 - protein, 119 aa, artificial sequence
  hH2L1, VH
EVQLQESGPGLVKPSETLSLTCTVSGFSLIDYGVSWIRQPPGKGLEWIGVIWGGGKIYYNSVLKSRVTISKDNSKSQVSLKLSSVTAADTAVYYCAKQGGLLFYAMDYWGQGTLVTVSS

SEQ ID NO: 6 - protein, 113 aa, artificial sequence
  hH2L1, VL
DIVMTQSPDSLAVSLGERATINCKSSQSLLNTYSQKNYLAWYQQKPGQPPKLLIYFASTRESGVPDRFSGSGSGTDFTLTISSLQAEDVAVYYCQQHYNTPFTFGGGTKVEIK

SEQ ID NO: 7 - protein, 119 aa, artificial sequence
  hL2H1mut1, VH
EVQLQESGPGLVKPSETLSLTCTVSGFSLIDYGVSWIRQPPGKGLEWIGVIWGGGKIYYNSVLKSRVTISVDTSKNQFSLKLSSVTAADTAVYYCAKQGGLLFYAMDYWGQGTLVTVSS

SEQ ID NO: 8 - protein, 113 aa, artificial sequence
  hL2H1mut1, VL
DIVMTQSPDSLAVSLGERATINCKSSQSLLNTYSQKNYLAWYQQKPGQSPKLLIYFASTRESGVPDRFSGSGSETDFTLTISSLQAEDLAVYFCQQHYNTPFTFGGGTKVEIK

SEQ ID NO: 9 - protein, 330 aa, artificial sequence
  CH
ASTKGPSVFPLAPSSKSTSGGTAALGCLVKDYFPEPVTVSWNSGALTSGVHTFPAVLQSSGLYSLSSVVTVPSSSLGTQTYICNVNHKPSNTKVDKRVEPKSCDKTHTCPPCPAPELLGGPSVFLFPPKPKDTLMISRTPEVTCVVVDVSHEDPEVKFNWYVDGVEVHNAKTKPREEQYNSTYRVVSVLTVLHQDWLNGKEYKCKVSNKALPAPIEKTISKAKGQPREPQVYTLPPSREEMTKNQVSLTCLVKGFYPSDIAVEWESNGQPENNYKTTPPVLDSDGSFFLYSKLTVDKSRWQQGNVFSCSVMHEALHNHYTQKSLSLSPGK

SEQ ID NO: 10 - protein, 107 aa, artificial sequence [sequence omitted]

SEQ ID NO: 11 - protein, 7 aa, artificial sequence
  CDR-H1
GFSLIDY

SEQ ID NO: 12 - protein, 5 aa, artificial sequence
  CDR-H2
WGGGK

SEQ ID NO: 13 - protein, 11 aa, artificial sequence
  CDR-H3
QGGLLFYAMDY

SEQ ID NO: 14 - protein, 17 aa, artificial sequence
  CDR-L1
KSSQSLLNTYSQKNYLA

SEQ ID NO: 15 - protein, 7 aa, artificial sequence
  CDR-L2
FASTRES

SEQ ID NO: 16 - protein, 9 aa, artificial sequence
  CDR-L3
QQHYNTPFT

SEQ ID NO: 17 - protein, 5 aa, artificial sequence
  CDR-H2
WGDGK

SEQ ID NO: 18 - protein, 17 aa, artificial sequence
  CDR-L1
KSSQSLLNSYSQKNYLA

SEQ ID NO: 19 - protein, 5 aa, artificial sequence
  CDR-H1
DYGVS

SEQ ID NO: 20 - protein, 16 aa, artificial sequence
  CDR-H2
VIWGGGKIYYNSVLKS